European Patent Application EP 4 679 092 A1, published January 14, 2026. Title: Biomarkers for Herpes-simplex virus autoimmunity. Applicant: Charité– Universitätsmedizin Berlin. Application EP. The sequence listing filed with the application follows.

SEQUENCE LISTING (7 sequences)

SEQ ID NO: 1 - protein, 96 aa, Human alphaherpesvirus 1
TKRGRSGGEDARADTALKKPKTGSPTAPPPADPVPLDTEDDSDAADGTAARPAAPDARSGSRYACYFRDLPTGEASPGAFSAFRGGPQTPYGFGFP

SEQ ID NO: 2 - protein, 84 aa, Human alphaherpesvirus 1
MVLIRAKLDSYSSFTTSPSEAVMREHAYSRARTKNNYGSTIEGLLDLPDDDAPEEAGLAAPRLSFLPAGHTRRLSTAPPTDVSL

SEQ ID NO: 3 - protein, 56 aa, Human alphaherpesvirus 1
TKRGRSGGEDARADTALKKPKTGSPTAPPPADPVPLDTEDDSDAADGTAARPAAPD

SEQ ID NO: 4 - protein, 56 aa, Human alphaherpesvirus 1
PPADPVPLDTEDDSDAADGTAARPAAPDARSGSRYACYFRDLPTGEASPGAFSAFR

SEQ ID NO: 5 - protein, 40 aa, Human alphaherpesvirus 1
ARSGSRYACYFRDLPTGEASPGAFSAFRGGPQTPYGFGFP

SEQ ID NO: 6 - protein, 56 aa, Human alphaherpesvirus 1
MVLIRAKLDSYSSFTTSPSEAVMREHAYSRARTKNNYGSTIEGLLDLPDDDAPEEA

SEQ ID NO: 7 - protein, 56 aa, Human alphaherpesvirus 1
SRARTKNNYGSTIEGLLDLPDDDAPEEAGLAAPRLSFLPAGHTRRLSTAPPTDVSL